European Patent Specification EP 3 625 331 B1, published July 10, 2024. Title: SYSTEMS AND METHODS FOR GROWTH OF INTESTINAL CELLS. Applicant: CEDARS-SINAI MEDICAL CENTER BARRETT, Robert SVENDSEN, Clive TARGAN, Stephan R. WORKMAN, Michael SAREEN, Dhruv RAJAMANI, Uthra. The sequence listing filed with the application follows.

SEQUENCE LISTING (12 sequences)

SEQ ID NO: 1 - DNA, 20 bp, Artificial Sequence
  IDO1 F
acactttgctaaaggcgctg

SEQ ID NO: 2 - DNA, 20 bp, Artificial Sequence
  IDO R
tgcctttccagccagacaaa

SEQ ID NO: 3 - DNA, 22 bp, Artificial Sequence
  GBP1 F
aaacttcaggaacaggagcaac

SEQ ID NO: 4 - DNA, 21 bp, Artificial Sequence
  GBP1 R
ggtacatgcctttcgtcgtct

SEQ ID NO: 5 - DNA, 20 bp, Artificial Sequence
  PLA2G2A F
caagtttagcaactcgggga

SEQ ID NO: 6 - DNA, 20 bp, Artificial Sequence
  PLA2G2A R
tctagcaaaacaggtggcag

SEQ ID NO: 7 - DNA, 19 bp, Artificial Sequence
  Muc4 F
agacgcacagccacatcac

SEQ ID NO: 8 - DNA, 20 bp, Artificial Sequence
  Muc4 R
gggaaactcctctctcaggc

SEQ ID NO: 9 - DNA, 20 bp, Artificial Sequence
  Lysozyme F
tttctgttacggtccagggc

SEQ ID NO: 10 - DNA, 21 bp, Artificial Sequence
  Lysozyme R
acacatccagtttgctaggct

SEQ ID NO: 11 - DNA, 21 bp, Artificial Sequence
  Reg3F
cctttagtgacccgattgcct

SEQ ID NO: 12 - DNA, 23 bp, Artificial Sequence
  Reg3R
tcttcaccttgaacctgacacag